European Patent Application EP 4 636 081 A2, published October 22, 2025. Title: Methods for Making L-Glufosinate. Applicant: BASF SE. The sequence listing filed with the application follows.

SEQUENCE LISTING (2 sequences)

SEQ ID NO: 1 - protein, 458 aa, Sinorhizobium arboris
MNIAAQSWERREATSFFHTFTDLPSLKTDGPVIIDHGEGPYIIDTVGRRYFEGNSGLWNMTLGFSERRLSDAALKQYQEFPGYHTFFGRNSKPTVELAERMLKLAPAPMSRVFFTNSGSEANESIVKLLWMMWAAEGRPERRKLLTRKNAYHGATVMASALTGKDYVKAFGLPGPEIVTLDCPHAWRFALPGEGDDEFAARLAANLETRILQEGPETIAGMFAEPVMGAGGVIVPPATYFAKIQPVLQRYGIPLIADEVICGFGRTGSLWGTLAVGQQPDIIVASKSMSAGYFPMGAVMLSADIDKRATAASEVWEEFPHGFTTGGHPVGCAISLEAIRIITEEGVFENVKSVSETFQSGLRALADHPMIGEARGMGLMGALETVADKKTKQSFSGDLRIGERISKEARDRGFIIRPLGSSVVLAPPFISTHGQIEELLAVLKEVLDVVYGTVKGEVA

SEQ ID NO: 2 - protein, 368 aa, Rhodosporidium toruloides
MHSQKRVVVLGSGVIGLSSALILARKGYSVHILARDLPEDVSSQTFASPWAGANWTPFMTLTDGPRQAKWEESTFKKWVELVPTGHAMWLKGTRRFAQNEDGLLGHWYKDITPNYRPLPSSECPPGAIGVTYDTLSVHAPKYCQYLARELQKLGATFERRTVTSLEQAFDGADLVVNATGLGAKSIAGIDDQAAEPIRGQTVLVKSPCKRCTMDSSDPASPAYIIPRPGGEVICGGTYGVGDWDLSVNPETVQRILKHCLRLDPTISSDGTIEGIEVLRHNVGLRPARRGGPRVEAERIVLPLDRTKSPLSLGRGSARAAKEKEVTLVHAYGFSSAGYQQSWGAAEDVAQLVDEAFQRYHGAARESKL